European Patent Application EP 4 174 865 A1, published May 3, 2023. Title: CONTROL METHOD AND ANALYSIS SYSTEM. Applicant: SYSMEX CORPORATION. Application EP. The sequence listing filed with the application follows.

SEQUENCE LISTING (4 sequences)

SEQ ID NO: 1 - DNA, 23 bp, Homo sapiens
  source 1..23: mol_type = other DNA
gccatggacagaaggcgcagggc

SEQ ID NO: 2 - DNA, 19 bp, Homo sapiens
  source 1..19: mol_type = other DNA
gccatggacagaaggcgca

SEQ ID NO: 3 - DNA, 16 bp, Homo sapiens
  source 1..16: mol_type = other DNA
gccatgcacagaaggc

SEQ ID NO: 4 - DNA, 19 bp, Homo sapiens
  source 1..19: mol_type = other DNA
gccatggacagtaggcgca